European Patent Specification EP 3 698 803 B1, published March 8, 2023. Title: METHODS OF TRANSDIFFERENTION AND METHODS OF USE THEREOF. Applicant: Orgenesis Ltd.; Tel HaShomer Medical Research Infrastructure and Services Ltd. The sequence listing filed with the application follows.

SEQUENCE LISTING (9 sequences)

SEQ ID NO: 1 - DNA, 51 bp, Rattus rattus - Artificial
tcacatggaaggatcaaagcaagcctgcttctattcttggaaacagagcaa

SEQ ID NO: 2 - DNA, 51 bp, Mus musculus - Artificial
tcacatgaaaggatcaaagcaaatccgcttctattcttggaaacagagcaa

SEQ ID NO: 3 - DNA, 51 bp, Homo sapiens - Artificial
tcacatgaatggatcaaagcaaatccatttccattcttggaaaagcagctc

SEQ ID NO: 4 - protein, 283 aa, Homo sapiens
MNGEEQYYAATQLYKDPCAFQRGPAPEFSASPPACLYMGRQPPPPPPHPFPGALGALEQGSPPDISPYEVPPLADDPAVAHLHHHLPAQLALPHPPAGPFPEGAEPGVLEEPNRVQLPFPWMKSTKAHAWKGQWAGGAYAAEPEENKRTRTAYTRAQLLELEKEFLFNKYISRPRRVELAVMLNLTERHIKIWFQNRRMKWKKEEDKKRGGGTAVGGGGVAEPEQDCAVTSGEELLALPPPPPPGGAVPPAAPVAAREGRLPPGLSASPQPSSVAPRRPQEPR

SEQ ID NO: 5 - DNA, 852 bp, Homo sapiens
atgaacggcgaggagcagtactacgcggccacgcagctttacaaggacccatgcgcgttccagcgaggcccggcgccggagttcagcgccagcccccctgcgtgcctgtacatgggccgccagcccccgccgccgccgccgcacccgttccctggcgccctgggcgcgctggagcagggcagccccccggacatctccccgtacgaggtgccccccctcgccgacgaccccgcggtggcgcaccttcaccaccacctcccggctcagctcgcgctcccccacccgcccgccgggcccttcccggagggagccgagccgggcgtcctggaggagcccaaccgcgtccagctgcctttcccatggatgaagtctaccaaagctcacgcgtggaaaggccagtgggcaggcggcgcctacgctgcggagccggaggagaacaagcggacgcgcacggcctacacgcgcgcacagctgctagagctggagaaggagttcctattcaacaagtacatctcacggccgcgccgggtggagctggctgtcatgttgaacttgaccgagagacacatcaagatctggttccaaaaccgccgcatgaagtggaaaaaggaggaggacaagaagcgcggcggcgggacagctgtcgggggtggcggggtcgcggagcctgagcaggactgcgccgtgacctccggcgaggagcttctggcgctgccgccgccgccgccccccggaggtgctgtgccgcccgctgcccccgttgccgcccgagagggccgcctgccgcctggccttagcgcgtcgccacagccctccagcgtcgcgcctcggcggccgcaggaaccacgatga

SEQ ID NO: 6 - protein, 356 aa, Homo sapiens
MTKSYSESGLMGEPQPQGPPSWTDECLSSQDEEHEADKKEDDLETMNAEEDSLRNGGEEEDEDEDLEEEEEEEEEDDDQKPKRRGPKKKKMTKARLERFKLRRMKANARERNRMHGLNAALDNLRKVVPCYSKTQKLSKIETLRLAKNYIWALSEILRSGKSPDLVSFVQTLCKGLSQPTTNLVAGCLQLNPRTFLPEQNQDMPPHLPTASASFPVHPYSYQSPGLPSPPYGTMDSSHVFHVKPPPHAYSAALEPFFESPLTDCTSPSFDGPLSPPLSINGNFSFKHEPSAEFEKNYAFTMHYPAATLAGAQSHGSIFSGTAAPRCEIPIDNIMSFDSHSHHERVMSAQLNAIFHD

SEQ ID NO: 7 - DNA, 1071 bp, Homo sapiens
atgaccaaatcgtacagcgagagtgggctgatgggcgagcctcagccccaaggtcctccaagctggacagacgagtgtctcagttctcaggacgaggagcacgaggcagacaagaaggaggacgacctcgaagccatgaacgcagaggaggactcactgaggaacgggggagaggaggaggacgaagatgaggacctggaagaggaggaagaagaggaagaggaggatgacgatcaaaagcccaagagacgcggccccaaaaagaagaagatgactaaggctcgcctggagcgttttaaattgagacgcatgaaggctaacgcccgggagcggaaccgcatgcacggactgaacgcggcgctagacaacctgcgcaaggtggtgccttgctattctaagacgcagaagctgtccaaaatcgagactctgcgcttggccaagaactacatctgggctctgtcggagatctcgcgctcaggcaaaagcccagacctggtctccttcgttcagacgctttgcaagggcttatcccaacccaccaccaacctggttgcgggctgcctgcaactcaatcctcggacttttctgcctgagcagaaccaggacatgcccccgcacctgccgacggccagcgcttccttccctgtacacccctactcctaccagtcgcctgggctgcccagtccgccttacggtaccatggacagctcccatgtcttccacgttaagcctccgccgcacgcctacagcgcagcgctggagcccttctttgaaagccctctgactgattgcaccagcccttcctttgatggacccctcagcccgccgctcagcatcaatggcaacttctctttcaaacacgaaccgtccgccgagtttgagaaaaattatgcctttaccatgcactatcctgcagcgacactggcaggggcccaaagccacggatcaatcttctcaggcaccgctgcccctcgctgcgagatccccatagacaatattatgtccttcgatagccattcacatcatgagcgagtcatgagtgcccagctcaatgccatatttcatgattag

SEQ ID NO: 8 - protein, 353 aa, Homo sapiens
MAAELAMGAELPSSPLAIEYVNDFDLMKFEVKKEPPEAERFCHRLPPGSLSSTPLSTPCSSVPSSPSFCAPSPGTGGGGGAGGGGGSSQAGGAPGPPSGGPGAVGGTSGKPALEDLYWMSGYQHHLNPEALNLTPEDAVEALIGSGHHGAHHGAHHPAAAAAYEAFRGPGFAGGGGADDMGAGHHHGAHHAAHHHHAAHHHHHHHHHHGGAGHGGGAGHHVRLEERFSDDQLVSMSVRELNRQLRGFSKEEVIRLKQKRRTLKNRGYAQSCRFKRVQQRHILESEKCQLQSQVEQLKLEVGRLAKERDLYKEKYEKLAGRGGPGSAGGAGFPREPSPPQAGPGGAKGTADFFL

SEQ ID NO: 9 - DNA, 1059 bp, Homo sapiens
atggccgcggagctggcgatgggcgccgagctgcccagcagcccgctggccatcgagtacgtcaacgacttcgacctgatgaagttcgaggtgaagaaggagcctcccgaggccgagcgcttctgccaccgcctgccgccaggctcgctgtcctcgacgccgctcagcacgccctgctcctccgtgccctcctcgcccagcttctgcgcgcccagcccgggcaccggcggcggcggcggcgcggggggcggcggcggctcgtctcaggccgggggcgcccccgggccgccgagcgggggccccggcgccgtcgggggcacctcggggaagccggcgctggaggatctgtactggatgagcggctaccagcatcacctcaaccccgaggcgctcaacctgacgcccgaggacgcggtggaggcgctcatcggcagcggccaccacggcgcgcaccacggcgcgcaccacccggcggccgccgcagcctacgaggctttccgcggcccgggcttcgcgggcggcggcggagcggacgacatgggcgccggccaccaccacggcgcgcaccacgccgcccaccaccaccacgccgcccaccaccaccaccaccaccaccaccatggcggcgcgggacacggcggtggcgcgggccaccacgtgcgcctggaggagcgcttctccgacgaccagctggtgtccatgtcggtgcgcgagctgaaccggcagctccgcggcttcagcaaggaggaggtcatccggctcaagcagaagcggcgcacgctcaagaaccgcggctacgcgcagtcctgccgcttcaagcgggtgcagcagcggcacattctggagagcgagaagtgccaactccagagccaggtggagcagctgaagctggaggtggggcgcctggccaaagagcgggacctgtacaaggagaaatacgagaagctggcgggccggggcggccccgggagcgcgggcggggccggtttcccgcgggagccttcgccgccgcaggccggtcccggcggggccaagggcacggccgacttcttcctgtag